European Patent Application EP 4 513 187 A2, published February 26, 2025. Title: Methods of Detecting Prostrate Cancer. Applicant: IMMUNIS.AI, INC. Application US. The sequence listing filed with the application follows.

SEQUENCE LISTING (4 sequences)

SEQ ID NO: 1 - DNA, 23 bp, synthetic construct
  misc_feature 1..23: note = Description of Artificial Sequence: Synthetic primer
  source 1..23: mol_type = other DNA
cagtgtgaaacgggagaaaacag

SEQ ID NO: 2 - DNA, 22 bp, synthetic construct
  misc_feature 1..22: note = Description of Artificial Sequence: Synthetic primer
  source 1..22: mol_type = other DNA
acttcgctgcagagtaccgaag

SEQ ID NO: 3 - DNA, 22 bp, synthetic construct
  misc_feature 1..22: note = Description of Artificial Sequence: Synthetic primer
  source 1..22: mol_type = other DNA
caatcagagacattccctctgg

SEQ ID NO: 4 - DNA, 20 bp, synthetic construct
  misc_feature 1..20: note = Description of Artificial Sequence: Synthetic primer
  source 1..20: mol_type = other DNA
agtggtcctctctgaatctc